European Patent Application EP 4 292 604 A1, published December 20, 2023. Title: Prophylactic administration for respiratory virus comprising administrating interferon beta to a subject potentially infected by respiratory virus. Applicant: ABION Inc. The sequence listing filed with the application follows.

SEQUENCE LISTING (4 sequences)

SEQ ID NO: 1 - protein, 166 aa, Artificial Sequence
  Human interferon beta R27T mutein (ABN101)
MSYNLLGFLQRSSNFQCQKLLWQLNGTLEYCLKDRMNFDIPEEIKQLQQFQKEDAALTIYEMLQNIFAIFRQDSSSTGWNETIVENLLANVYHQINHLKTVLEEKLEKEDFTRGKLMSSLHLKRYYGRILHYLKAKEYSHCAWTIVRVEILRNFYFINRLTGYLRN

SEQ ID NO: 2 - DNA, 22 bp, Artificial Sequence
  SARS-CoV-2  E gene probe sequence
atattgcagcagtacgcacaca

SEQ ID NO: 3 - DNA, 26 bp, Artificial Sequence
  SARS-CoV-2  E gene primer-1 sequence
acaggtacgttaatagttaatagcgt

SEQ ID NO: 4 - DNA, 22 bp, Artificial Sequence
  SARS-CoV-2  E gene primer-2 sequence
atattgcagcagtacgcacaca